European Patent Application EP 4 710 937 A1, published March 18, 2026. Title: Pharmaceutical Composition. Applicant: National University Corporation Kumamoto University. Application JP. The sequence listing filed with the application follows.

SEQUENCE LISTING (33 sequences)

SEQ ID NO: 1 - protein, 429 aa, Human T-cell leukemia virus type 1
MGQIFSRSASPIPRPPRGLAAHHWLNFLQAAYRLEPGPSSYDFHQLKKFLKIALETPVWICPINYSLLASLLPKGYPGRVNEILHILIQTQAQIPSRPAPPPPSSPTHDPPDSDPQIPPPYVEPTAPQVLPVMHPHGAPPNHRPWQMKDLQAIKQEVSQAAPGSPQFMQTIRLAVQQFDPTAKDLQDLLQYLCSSLVASLHHQQLDSLISEAETRGITGYNPLAGPLRVQANNPQQQGLRREYQQLWLAAFAALPGSAKDPSWASILQGLEEPYHAFVERLNIALDNGLPEGTPKDPILRSLAYSNANKECQKLLQARGHTNSPLGDMLRACQTWTPKDKTKVLVVQPKKPPPNQPCFRCGKAGHWSRDCTQPRPPPGPCPLCQDPTHWKRDCPRLKPTIPEPEPEEDALLLDLPADIPHPKNSIGGEV

SEQ ID NO: 2 - DNA, 1290 bp, Human T-cell leukemia virus type 1
  source 1..1290: mol_type = genomic DNA
atgggccaaatcttttcccgtagcgctagccctattccgcggccgccccgggggctggccgctcatcactggcttaacttcctccaggcggcatatcgcctagaacccggtccctccagttacgatttccaccagttaaaaaaatttcttaaaatagctttagaaacaccagtctggatctgtcccattaactactccctcctagccagcctactcccaaaaggataccccggccgggtgaatgaaattttacacatactcatccaaacccaagcccagatcccgtcccgtcccgcgccaccgccgccgtcatcccccacccacgaccccccggattctgatccacaaatcccccctccctatgttgagcctacggccccccaagtccttccagtcatgcacccacatggtgcccctcccaaccatcgcccatggcaaatgaaagacctacaggccattaagcaagaagtctcccaagcagcccctgggagcccccagtttatgcagaccatccggcttgcggtgcagcagtttgaccccactgccaaagacctccaagacctcctgcagtacctttgctcctccctcgtggcttccctccatcaccagcagctagatagccttatatcagaggccgaaacccgaggtattacaggttataaccccttagccggtcccctccgtgtccaagccaacaatccacaacaacaaggattaaggcgagaataccagcaactctggctcgccgccttcgccgccctgccggggagtgccaaagacccttcctgggcctctatcctccaaggcctggaggagccttaccacgccttcgtagaacgcctcaacatagctcttgacaatgggctgccagaaggcacgcccaaagaccccatcttacgttccttagcctactccaatgcaaacaaagaatgccaaaaattactacaggcccgaggacacactaatagccctctaggagatatgttgcgggcttgtcagacctggacccccaaagacaaaaccaaagtgttagttgtccagcctaaaaaaccccccccaaatcagccgtgcttccggtgcgggaaagcaggccactggagtcgggactgcactcagcctcgccccccccccgggccatgccccctatgtcaagacccaactcactggaagcgagactgcccccgcctaaagcccactatcccagaaccagagccagaggaagatgccctcctattagacctccccgctgacatcccacacccaaaaaactccatagggggggaggtttaa

SEQ ID NO: 3 - protein, 353 aa, Human T-cell leukemia virus type 1
MAHFPGFGQSLLFGYPVYVFGDCVQGDWCPISGGLCSARLHRHALLATCPEHQITWDPIDGRVIGSALQFLIPRLPSFPTQRTSKTLKVLTPPITHTTPNIPPSFLQAMRKYSPFRNGYMEPTLGQHLPTLSFPDPGLRPQNLYTLWGGSVVCMYLYQLSPPITWPLLPHVIFCHPGQLGAFLTNVPYKRIEELLYKISLTTGALIILPEDCLPTTLFQPARAPVTLTAWQNGLLPFHSTLTTPGLIWTFTDGTPMISGPCPKDGQPSLVLQSSSFIFHKFQTKAYHPSFLLSHGLIQYSSFHSLHLLFEEYTNIPISLLFNEKEADDNDHEPQISPGGLEPPSEKHFRETEV

SEQ ID NO: 4 - DNA, 1062 bp, Human T-cell leukemia virus type 1
  source 1..1062: mol_type = genomic DNA
atggcccacttcccagggtttggacagagtcttcttttcggatacccagtctacgtgtttggagactgtgtacaaggcgactggtgccccatctctgggggactatgttcggcccgcctacatcgtcacgccctactggccacctgtccagagcatcagatcacctgggaccccatcgatggacgcgttatcggctcagctctacagttccttatccctcgactcccctccttccccacccagagaacctctaagaccctcaaggtccttaccccgccaatcactcatacaacccccaacattccaccctccttcctccaggccatgcgcaaatactcccccttccgaaatggatacatggaaccaacccttgggcagcacctcccaaccctgtcttttccagaccccggactccggccccaaaacctgtacaccctctggggaggctccgttgtctgcatgtacctctaccagctttccccccccatcacctggcccctcctgccccacgtgattttttgccaccccggccagctcggggccttcctcaccaatgttccctacaagcgaatagaagaactcctctataaaatttccctcaccacaggggccctaataattctacccgaagactgtttgcccaccacccttttccagcctgctagggcacccgtcacgctaacagcctggcaaaacggcctccttccgttccactcaaccctcaccactccaggccttatttggacatttaccgatggcacgcctatgatttccgggccctgccctaaagatggccagccatctttagtactacagtcctcctcctttatatttcacaaatttcaaaccaaggcctaccacccctcatttctactctcacacggcctcatacagtactcttcctttcatagtttacatctcctgtttgaagaatacaccaacatccccatttctctactttttaacgaaaaagaggcagatgacaatgaccatgagccccaaatatcccccgggggcttagagcctcccagtgaaaaacatttccgagaaacagaagtctga

SEQ ID NO: 5 - protein, 206 aa, Human T-cell leukemia virus type 1
MAASGLFRCLPVSCPEDLLVEELVDGLLSLEEELKDKEEEEAVLDGLLSLEEESRGRLRRGPPGEKAPPRGETHRDRQRRAEEKRKRKKEREKEEEKQTAEYLKRKEEEKARRRRRAEKKAADVARRKQEEQERRERKWRQGAEKAKQHSARKEKMQELGIDGYTRQLEGEVESLEAERRKLLQEKEDLMGEVNYWQGRLEAMWLQ

SEQ ID NO: 6 - DNA, 621 bp, Human T-cell leukemia virus type 1
  source 1..621: mol_type = genomic DNA
atggcggcctcagggctgtttcgatgcttgcctgtgtcatgcccggaggacctgctggtggaggaattggtggacgggctattatccttggaggaagagttaaaggacaaggaggaggaggaagctgtgcttgacggtttgctatccttagaagaggaaagccgcggccggctgcgacggggccctccaggggagaaagcgccacctcgcggggaaacgcatcgtgatcggcagcgacgggctgaggagaagaggaagcgaaaaaaagagcgggagaaagaggaggaaaagcagaccgctgagtatttgaaaaggaaggaagaggagaaggcacggcgcaggaggcgggcggagaagaaggccgctgacgtcgctaggaggaagcaggaagagcaggagcgccgtgagcgcaagtggagacaaggggctgagaaggcgaaacagcatagtgctaggaaagaaaaaatgcaggagttggggattgatggctatactagacagttggaaggcgaggtggagtccttggaggctgaacggaggaagttgctgcaggagaaggaggatttgatgggagaggttaattattggcaggggaggctggaggcgatgtggttgcaataa

SEQ ID NO: 7 - protein, 206 aa, Human T-cell leukemia virus type 1
MAASGLFRCLPVSCPEDLLVEELVDGLLSLEEELKDKEEEEAVLDGLLSLEEESRGRLRRGPPGEKAPPRGETHRDRQRRAEEKRKRKKEREKEEEKQIAEYLKRKEEEKARRRRRAEKKAADVARRKQEEQERRERKWRQGAEKAKQHSARKEKMQELGIDGYTRQLEGEVESLEAERRKLLQEKEDLMGEVNYWQGRLEAMWLQ

SEQ ID NO: 8 - DNA, 621 bp, Human T-cell leukemia virus type 1
  source 1..621: mol_type = genomic DNA
atggcggcctcagggctgtttcgatgcttgcctgtgtcatgcccggaggacctgctggtggaggaattggtggacgggctattatccttggaggaagagttaaaggacaaggaggaggaggaagctgtgcttgacggtttgctatccttagaagaggaaagccgcggccggctgcgacggggccctccaggggagaaagcgccacctcgcggggaaacgcatcgtgatcggcagcgacgggccgaggagaagaggaagcgaaaaaaagagcgggagaaagaggaggaaaagcagattgctgagtatttgaaaaggaaggaagaggagaaggcacggcgcaggaggcgggcggagaagaaggccgctgacgtcgccaggaggaagcaggaagagcaggagcgccgtgagcgcaagtggagacaaggggctgagaaggcgaaacagcatagtgctaggaaagaaaaaatgcaggagttggggattgatggctatactagacagttggaaggcgaggtggagtccttggaggctgaacggaggaagttgctgcaggagaaggaggatttgatgggagaggttaattattggcaggggaggctggaggcgatgtggttgcaataa

SEQ ID NO: 9 - protein, 105 aa, Human T-cell leukemia virus type 1
VVQPKKPPPNQPCFRCGKAGHWSRDCTQPRPPPGPCPLCQDPTHWKRDCPRLKPTIPEPEPEEDALLLDLPADIPHPKNLHRGGGLTSPPTLQQVLPNQDPASIL

SEQ ID NO: 10 - protein, 85 aa, Human T-cell leukemia virus type 1
VVQPKKPPPNQPCFRCGKAGHWSRDCTQPRPPPGPCPLCQDPTHWKRDCPRLKPTIPEPEPEEDALLLDLPADIPHPKNSIGGEV

SEQ ID NO: 11 - protein, 130 aa, Human T-cell leukemia virus type 1
MGQIFSRSASPIPRPPRGLAAHHWLNFLQAAYRLEPGPSSYDFHQLKKFLKIALETPVWICPINYSLLASLLPKGYPGRVNEILHILIQTQAQIPSRPAPPPPSSPTHDPPDSDPQIPPPYVEPTAPQVL

SEQ ID NO: 12 - protein, 214 aa, Human T-cell leukemia virus type 1
PVMHPHGAPPNHRPWQMKDLQAIKQEVSQAAPGSPQFMQTIRLAVQQFDPTAKDLQDLLQYLCSSLVASLHHQQLDSLISEAETRGITGYNPLAGPLRVQANNPQQQGLRREYQQLWLAAFAALPGSAKDPSWASILQGLEEPYHAFVERLNIALDNGLPEGTPKDPILRSLAYSNANKECQKLLQARGHTNSPLGDMLRACQTWTPKDKTKVL

SEQ ID NO: 13 - DNA, 315 bp, Human T-cell leukemia virus type 1
  source 1..315: mol_type = genomic DNA
gttgtccagcctaaaaaaccccccccaaatcagccgtgcttccggtgcgggaaagcaggccactggagtcgggactgcactcagcctcgccccccccccgggccatgccccctatgtcaagacccaactcactggaagcgagactgcccccgcctaaagcccactatcccagaaccagagccagaggaagatgccctcctattagacctccccgctgacatcccacacccaaaaaacctccatagggggggaggtttaacctccccccccacattacagcaagtccttcctaaccaagacccagcatctattctg

SEQ ID NO: 14 - DNA, 255 bp, Human T-cell leukemia virus type 1
  source 1..255: mol_type = genomic DNA
gttgtccagcctaaaaaaccccccccaaatcagccgtgcttccggtgcgggaaagcaggccactggagtcgggactgcactcagcctcgccccccccccgggccatgccccctatgtcaagacccaactcactggaagcgagactgcccccgcctaaagcccactatcccagaaccagagccagaggaagatgccctcctattagacctccccgctgacatcccacacccaaaaaactccatagggggggaggtt

SEQ ID NO: 15 - DNA, 387 bp, Human T-cell leukemia virus type 1
  source 1..387: mol_type = genomic DNA
ggccaaatcttttcccgtagcgctagccctattccgcggccgccccgggggctggccgctcatcactggcttaacttcctccaggcggcatatcgcctagaacccggtccctccagttacgatttccaccagttaaaaaaatttcttaaaatagctttagaaacaccagtctggatctgtcccattaactactccctcctagccagcctactcccaaaaggataccccggccgggtgaatgaaattttacacatactcatccaaacccaagcccagatcccgtcccgtcccgcgccaccgccgccgtcatcccccacccacgaccccccggattctgatccacaaatcccccctccctatgttgagcctacggccccccaagtcctt

SEQ ID NO: 16 - DNA, 642 bp, Human T-cell leukemia virus type 1
  source 1..642: mol_type = genomic DNA
ccagtcatgcacccacatggtgcccctcccaaccatcgcccatggcaaatgaaagacctacaggccattaagcaagaagtctcccaagcagcccctgggagcccccagtttatgcagaccatccggcttgcggtgcagcagtttgaccccactgccaaagacctccaagacctcctgcagtacctttgctcctccctcgtggcttccctccatcaccagcagctagatagccttatatcagaggccgaaacccgaggtattacaggttataaccccttagccggtcccctccgtgtccaagccaacaatccacaacaacaaggattaaggcgagaataccagcaactctggctcgccgccttcgccgccctgccggggagtgccaaagacccttcctgggcctctatcctccaaggcctggaggagccttaccacgccttcgtagaacgcctcaacatagctcttgacaatgggctgccagaaggcacgcccaaagaccccatcttacgttccttagcctactccaatgcaaacaaagaatgccaaaaattactacaggcccgaggacacactaatagccctctaggagatatgttgcgggcttgtcagacctggacccccaaagacaaaaccaaagtgtta

SEQ ID NO: 17 - protein, 353 aa, Human T-cell leukemia virus type 1; identical to SEQ ID NO: 3

SEQ ID NO: 18 - protein, 488 aa, Human T-cell leukemia virus type 1
MGKFLATLILFFQFCPLIFGDYSPSCCTLTIGVSSYHSKPCNPAQPVCSWTLDLLALSADQALQPPCPNLVSYSSYHATYSLYLFPHWIKKPNRNGGGYYSASYSDPCSLKCPYLGCQSWTCPYTGAVSSPYWKFQHDVNFTQEVSRLNINLHFSKCGFPFSLLVDAPGYDPIWFLNTEPSQLPPTAPPLLPHSNLDHILEPSIPWKSKLLTLVQLTLQSTNYTCIVCIDRASLSTWHVLYSPNVSVPSSSSTPLLYPSLALPAPHLTLPFNWTHCFDPQIQAIVSSPCHNSLILPPFSLSPVPTLGSRSRRAVPVAVWLVSALAMGAGVAGGITGSMSLASGKSLLHEVDKDISQLTQAIVKNHKNLLKIAQYAAQNRRGLDLLFWEQGGLCKALQEQCCFLNITNSHVSILQERPPLENRVLTGWGLNWDLGLSQWAREALQTGITLVALLLLVILAGPCILRQLRHLPSRVRYPHYSLINPESSL

SEQ ID NO: 19 - protein, 105 aa, Human T-cell leukemia virus type 1; identical to SEQ ID NO: 9

SEQ ID NO: 20 - protein, 130 aa, Human T-cell leukemia virus type 1; identical to SEQ ID NO: 11

SEQ ID NO: 21 - protein, 214 aa, Human T-cell leukemia virus type 1; identical to SEQ ID NO: 12

SEQ ID NO: 22 - DNA, 15 bp, synthetic construct
  source 1..15: mol_type = other DNA; note = cDNA synthesis primer for Gag
tgcaggatatgggcc

SEQ ID NO: 23 - DNA, 20 bp, synthetic construct
  source 1..20: mol_type = other DNA; note = primer set for Gag
agtacctttgctcctccctc

SEQ ID NO: 24 - DNA, 20 bp, synthetic construct
  source 1..20: mol_type = other DNA; note = primer set for Gag
taatacctcgggtttcggcc

SEQ ID NO: 25 - DNA, 27 bp, synthetic construct
  source 1..27: mol_type = other DNA; note = probe for Gag
ttccctccatcaccagctagatagcct

SEQ ID NO: 26 - DNA, 17 bp, synthetic construct
  source 1..17: mol_type = other DNA; note = primer set for Tax
ccgccgatcccaaagaa

SEQ ID NO: 27 - DNA, 19 bp, synthetic construct
  source 1..19: mol_type = other DNA; note = primer set for Tax
cctgtccaaaccctgggaa

SEQ ID NO: 28 - DNA, 17 bp, synthetic construct
  source 1..17: mol_type = other DNA; note = T7 promoter
taatacgactcactata

SEQ ID NO: 29 - DNA, 41 bp, synthetic construct
  source 1..41: mol_type = other DNA; note = 5'UTR
aggaaataagagagaaaagaagagtaagaagaaatataaga

SEQ ID NO: 30 - skipped

SEQ ID NO: 31 - DNA, 100 bp, synthetic construct
  source 1..100: mol_type = other DNA; note = 3'UTR
taagctgccttctgcggggcttgccttctggccatgcccttcttctctcccttgcacctgtacctcttggtctttgaataaagcctgagtaggaaggcgg

SEQ ID NO: 32 - DNA, 1454 bp, Human T-cell leukemia virus type 1
  source 1..1454: mol_type = genomic DNA
taatacgactcactataaggaaataagagagaaaagaagagtaagaagaaatataagagccaccatgggccagatcttctctcgctctgcttctcctattcctcgccctcctcgcggacttgctgctcaccactggcttaacttcctgcaggctgcttaccgcctggaacctggccctagcagctacgacttccaccagctgaagaagttcctgaagatcgccctggagacccccgtgtggatctgccccatcaactacagcctgctggctagcctgctgcctaaaggctaccctggccgcgtgaacgagatcctgcacatcctgatccagacccaggcccagatcccttctcgccctgctcctcctcctccttcttctcctacccacgatccccccgatagcgatccccagatcccccctccttacgtggaacctaccgctcctcaggtgctgcctgtgatgcaccctcacggcgctcctcctaatcaccgcccttggcagatgaaggacctgcaggccatcaaacaggaagtgagccaggctgctcccggcagcccccagtttatgcagaccatccgcctggctgtgcagcagttcgatcccaccgctaaagatctgcaggacctgctgcagtacctgtgcagcagcctggtggctagcctgcaccaccagcagctggatagcctgatcagcgaagccgaaacccgcggcatcaccggctacaatcctctggctggccctctgcgcgtgcaggctaacaaccctcagcagcagggactgcgccgcgaataccagcagctgtggctggctgcttttgctgctctgcccggcagcgctaaagatcccagctgggctagcatcctgcagggcctggaagaaccctaccacgccttcgtggagcgcctgaacatcgccctggacaacggcctgcctgaaggcacccctaaagatcctatcctgcgcagcctggcctacagcaacgccaacaaggagtgccagaagctgctgcaggctcgcggacacaccaatagccctctgggagatatgctgcgcgcttgccagacctggacccccaaggacaagaccaaggtgctggtggtgcagcccaagaagcctcctcctaaccagccttgctttcgctgcggcaaagctggacactggagccgcgattgcacacagcctcgccctcctcctggaccttgccctctttgccaggatcctacccactggaagcgcgactgccctcgcctgaaacctaccatccctgaacctgaacctgaagaagacgctctgctgctggatctgcccgctgatatcccccaccccaagaacagcatcggcggcgaggtgtgataagctgccttctgcggggcttgccttctggccatgcccttcttctctcccttgcacctgtacctcttggtctttgaataaagcctgagtaggaaggcgg

SEQ ID NO: 33 - RNA, 1557 nt, Human T-cell leukemia virus type 1
  source 1..1557: mol_type = mRNA
aggaaataagagagaaaagaagagtaagaagaaatataagagccaccatgggccagatcttctctcgctctgcttctcctattcctcgccctcctcgcggacttgctgctcaccactggcttaacttcctgcaggctgcttaccgcctggaacctggccctagcagctacgacttccaccagctgaagaagttcctgaagatcgccctggagacccccgtgtggatctgccccatcaactacagcctgctggctagcctgctgcctaaaggctaccctggccgcgtgaacgagatcctgcacatcctgatccagacccaggcccagatcccttctcgccctgctcctcctcctccttcttctcctacccacgatccccccgatagcgatccccagatcccccctccttacgtggaacctaccgctcctcaggtgctgcctgtgatgcaccctcacggcgctcctcctaatcaccgcccttggcagatgaaggacctgcaggccatcaaacaggaagtgagccaggctgctcccggcagcccccagtttatgcagaccatccgcctggctgtgcagcagttcgatcccaccgctaaagatctgcaggacctgctgcagtacctgtgcagcagcctggtggctagcctgcaccaccagcagctggatagcctgatcagcgaagccgaaacccgcggcatcaccggctacaatcctctggctggccctctgcgcgtgcaggctaacaaccctcagcagcagggactgcgccgcgaataccagcagctgtggctggctgcttttgctgctctgcccggcagcgctaaagatcccagctgggctagcatcctgcagggcctggaagaaccctaccacgccttcgtggagcgcctgaacatcgccctggacaacggcctgcctgaaggcacccctaaagatcctatcctgcgcagcctggcctacagcaacgccaacaaggagtgccagaagctgctgcaggctcgcggacacaccaatagccctctgggagatatgctgcgcgcttgccagacctggacccccaaggacaagaccaaggtgctggtggtgcagcccaagaagcctcctcctaaccagccttgctttcgctgcggcaaagctggacactggagccgcgattgcacacagcctcgccctcctcctggaccttgccctctttgccaggatcctacccactggaagcgcgactgccctcgcctgaaacctaccatccctgaacctgaacctgaagaagacgctctgctgctggatctgcccgctgatatcccccaccccaagaacagcatcggcggcgaggtgtgataagctgccttctgcggggcttgccttctggccatgcccttcttctctcccttgcacctgtacctcttggtctttgaataaagcctgagtaggaaggcggaaaaaaaaaaaaaaaaaaaaaaaaaaaaaaaaaaaaaaaaaaaaaaaaaaaaaaaaaaaaaaaaaaaaaaaaaaaaaaaaaaaaaaaaaaaaaaaaaaaaaaaaaaaaaaaaaaaaaaaa